European Patent Application EP 4 148 138 A1, published March 15, 2023. Title: Process for the modification of a glycoprotein using a b-(1,4)-N-acetylgalactosaminyltransferase or a mutant thereof. Applicant: Synaffix B.V. The sequence listing filed with the application follows.

SEQUENCE LISTING (89 sequences)

SEQ ID NO: 1 - protein, 402 aa, synthetic construct
  REGION 1..402: note = Bos Taurus GalT Y289L mutant
MKFREPLLGGSAAMPGASLQRACRLLVAVCALHLGVTLVYYLAGRDLRRLPQLVGVHPPLQGSSHGAAAIGQPSGELRLRGVAPPPPLQNSSKPRSRAPSNLDAYSHPGPGPGPGSNLTSAPVPSTTTRSLTACPEESPLLVGPMLIEFNIPVDLKLIEQQNPKVKLGGRYTPMDCISPHKVAIIILFRNRQEHLKYWLYYLHPMVQRQQLDYGIYVINQAGESMFNRAKLLNVGFKEALKDYDYNCFVFSDVDLIPMNDHNTYRCFSQPRHISVAMDKFGFSLPYVQLFGGVSALSKQQFLSINGFPNNYWGWGGEDDDIYNRLAFRGMSVSRPNAVIGKCRMIRHSRDKKNEPNPQRFDRIAHTKETMLSDGLNSLTYMVLEVQRYPLYTKITVDIGTPS

SEQ ID NO: 2 - protein, 383 aa, Caenorhabditis elegans
MAFRHLAVARLKSLLVLCAVLLLVHAMIYKIPSLYENLTIGSSTLIADVDAMEAVLGNTASTSDDLLDTWNSTFSPISEVNQTSFMEDIRPILFPDNQTLQFCNQTPPHLVGPIRVFLDEPDFKTLEKIYPDTHAGGHGMPKDCVARHRVAIIVPYRDREAHLRIMLHNLHSLLAKQQLDYAIFIVEQVANQTFNRGKLMNVGYDVASRLYPWQCFIFHDVDLLPEDDRNLYTCPIQPRHMSVAIDKFNYKLPYSAIFGGISALTKDHLKKINGFSNDFWGWGGEDDDLATRTSMAGLKVSRYPTQIARYKMIKHSTEATNPVNKCRYKIMGQTKRRWTRDGLSNLKYKLVNLELKPLYTRAVVDLLEKDCRRELRRDFPTCF

SEQ ID NO: 3 - protein, 383 aa, Ascaris suum
MNSKLKLVIVLTLCVAIIHFLLSDCPISPDYSFWSPAFIISAPKTLTTLQPFSQSTSTNDLAVSALESVEFSMLDNSSILHASDNWTNDELVMRAQNENLQLCPMTPPALVGPIKVWMDAPSFAELERLYPFLEPGGHGMPTACRARHRVAIVVPYRDRESHLRTFLHNLHSLLTKQQLDYAIFVVEQTANETFNRAKLMNVGYAEAIRLYDWRCFIFHDVDLLPEDDRNLYSCPDEPRHMSVAVDKFNYKLPYGSIFGGISALTREQFEGINGFSNDYWGWGGEDDDLSTRVTLAGYKISRYPAEIARYKMIKHNSEKKNPVNRCRYKLMSATKSRWRNDGLSSLSYDLISLGRLPLYTHIKVDLLEKQSRRYLRTHGFPTC

SEQ ID NO: 4 - protein, 421 aa, Trichoplusia ni
MGGRATRALRLLLLLVLALAAVEYLFGSILDASPLRTYLYTPLYNATQPTLRNVERLAANWPKKIPSNYIEDSEEYSIKNISLSNHTTRASVVHPPSSITETASKLDKNMTIQDGAFAMISPTPLLITKLMDSIKSYVTTEDGVKKAEAVVTLPLCDSMPPDLGPITLNKTELELEWVEKKFPEVEWGGRYSPPNCTARHRVAIIVPYRDRQQHLAIFLNHMHPFLMKQQIEYGIFIVEQEGNKDFNRAKLMNVGFVESQKLVAEGWQCFVFHDIDLLPLDTRNLYSCPRQPRHMSASIDKLHFKLPYEDIFGGVSAMTLEQFTRVNGFSNKYWGWGGEDDDMSYRLKKINYHIARYKMSIARYAMLDHKKSTPNPKRYQLLSQTSKTFQKDGLSTLEYELVQVVQYHLYTHILVNIDERS

SEQ ID NO: 5 - protein, 403 aa, Drosophila melanogaster
MYLFTKANLIRFLAGAICLLLVLNFVGFRSDGGSATSLSKLSIRRVHKYAHIYGNASSDGAGGSEASRLPASPLALSKDRERDQELNGGPNSTIRTVIATANFTSIPQDLTRFLLGTKKFLPPRQKSTSALLANCTDPDPRDGGPITPNTTLESLDVIEAELGPLLRPGGAFEPENCNAQHHVAIVVPFRDRYAHLLLFLRNIHPFLMKQRIAYRIFIVEQTNGKPFNRAAMMNIGYLEALKLYQWDCFIFHDVDLLPLDDRNLYNCPRQPRHMSVAIDTLNFRLPYRSIFGGVSAMTREHFQAVNGFSNSFFGWGGEDDDMSNRLKHANLFISRYPVNIARYKMLKHQKEKANPKRYENLQNGMSKIEQDGINSIKYSIYSIKQFPTFTWYLAELKNSERKS

SEQ ID NO: 6 - protein, 354 aa, synthetic construct
  REGION 1..354: note = CeGalNAcT(30-383)
KIPSLYENLTIGSSTLIADVDAMEAVLGNTASTSDDLLDTWNSTFSPISEVNQTSFMEDIRPILFPDNQTLQFCNQTPPHLVGPIRVFLDEPDFKTLEKIYPDTHAGGHGMPKDCVARHRVAIIVPYRDREAHLRIMLHNLHSLLAKQQLDYAIFIVEQVANQTFNRGKLMNVGYDVASRLYPWQCFIFHDVDLLPEDDRNLYTCPIQPRHMSVAIDKFNYKLPYSAIFGGISALTKDHLKKINGFSNDFWGWGGEDDDLATRTSMAGLKVSRYPTQIARYKMIKHSTEATNPVNKCRYKIMGQTKRRWTRDGLSNLKYKLVNLELKPLYTRAVVDLLEKDCRRELRRDFPTCF

SEQ ID NO: 7 - protein, 354 aa, synthetic construct
  REGION 1..354: note = AsGalNAcT (30-383)
DYSFWSPAFIISAPKTLTTLQPFSQSTSTNDLAVSALESVEFSMLDNSSILHASDNWTNDELVMRAQNENLQLCPMTPPALVGPIKVWMDAPSFAELERLYPFLEPGGHGMPTACRARHRVAIVVPYRDRESHLRTFLHNLHSLLTKQQLDYAIFVVEQTANETFNRAKLMNVGYAEAIRLYDWRCFIFHDVDLLPEDDRNLYSCPDEPRHMSVAVDKFNYKLPYGSIFGGISALTREQFEGINGFSNDYWGWGGEDDDLSTRVTLAGYKISRYPAEIARYKMIKHNSEKKNPVNRCRYKLMSATKSRWRNDGLSSLSYDLISLGRLPLYTHIKVDLLEKQSRRYLRTHGFPTC

SEQ ID NO: 8 - protein, 389 aa, synthetic construct
  REGION 1..389: note = TnGalNAcT(33-421)
SPLRTYLYTPLYNATQPTLRNVERLAANWPKKIPSNYIEDSEEYSIKNISLSNHTTRASVVHPPSSITETASKLDKNMTIQDGAFAMISPTPLLITKLMDSIKSYVTTEDGVKKAEAVVTLPLCDSMPPDLGPITLNKTELELEWVEKKFPEVEWGGRYSPPNCTARHRVAIIVPYRDRQQHLAIFLNHMHPFLMKQQIEYGIFIVEQEGNKDFNRAKLMNVGFVESQKLVAEGWQCFVFHDIDLLPLDTRNLYSCPRQPRHMSASIDKLHFKLPYEDIFGGVSAMTLEQFTRVNGFSNKYWGWGGEDDDMSYRLKKINYHIARYKMSIARYAMLDHKKSTPNPKRYQLLSQTSKTFQKDGLSTLEYELVQVVQYHLYTHILVNIDERS

SEQ ID NO: 9 - protein, 357 aa, synthetic construct
  REGION 1..357: note = DmGalNAcT (47-403)
HKYAHIYGNASSDGAGGSEASRLPASPLALSKDRERDQELNGGPNSTIRTVIATANFTSIPQDLTRFLLGTKKFLPPRQKSTSALLANCTDPDPRDGGPITPNTTLESLDVIEAELGPLLRPGGAFEPENCNAQHHVAIVVPFRDRYAHLLLFLRNIHPFLMKQRIAYRIFIVEQTNGKPFNRAAMMNIGYLEALKLYQWDCFIFHDVDLLPLDDRNLYNCPRQPRHMSVAIDTLNFRLPYRSIFGGVSAMTREHFQAVNGFSNSFFGWGGEDDDMSNRLKHANLFISRYPVNIARYKMLKHQKEKANPKRYENLQNGMSKIEQDGINSIKYSIYSIKQFPTFTWYLAELKNSERKS

SEQ ID NO: 10 - protein, 354 aa, synthetic construct
  REGION 1..354: note = CeGalNacT(30-383; I257L)
KIPSLYENLTIGSSTLIADVDAMEAVLGNTASTSDDLLDTWNSTFSPISEVNQTSFMEDIRPILFPDNQTLQFCNQTPPHLVGPIRVFLDEPDFKTLEKIYPDTHAGGHGMPKDCVARHRVAIIVPYRDREAHLRIMLHNLHSLLAKQQLDYAIFIVEQVANQTFNRGKLMNVGYDVASRLYPWQCFIFHDVDLLPEDDRNLYTCPIQPRHMSVAIDKFNYKLPYSALFGGISALTKDHLKKINGFSNDFWGWGGEDDDLATRTSMAGLKVSRYPTQIARYKMIKHSTEATNPVNKCRYKIMGQTKRRWTRDGLSNLKYKLVNLELKPLYTRAVVDLLEKDCRRELRRDFPTCF

SEQ ID NO: 11 - protein, 354 aa, synthetic construct
  REGION 1..354: note = CeGalNAcT(30-383; I257M)
KIPSLYENLTIGSSTLIADVDAMEAVLGNTASTSDDLLDTWNSTFSPISEVNQTSFMEDIRPILFPDNQTLQFCNQTPPHLVGPIRVFLDEPDFKTLEKIYPDTHAGGHGMPKDCVARHRVAIIVPYRDREAHLRIMLHNLHSLLAKQQLDYAIFIVEQVANQTFNRGKLMNVGYDVASRLYPWQCFIFHDVDLLPEDDRNLYTCPIQPRHMSVAIDKFNYKLPYSAMFGGISALTKDHLKKINGFSNDFWGWGGEDDDLATRTSMAGLKVSRYPTQIARYKMIKHSTEATNPVNKCRYKIMGQTKRRWTRDGLSNLKYKLVNLELKPLYTRAVVDLLEKDCRRELRRDFPTCF

SEQ ID NO: 12 - protein, 354 aa, synthetic construct
  REGION 1..354: note = CeGalNacT(30-383; I257A)
KIPSLYENLTIGSSTLIADVDAMEAVLGNTASTSDDLLDTWNSTFSPISEVNQTSFMEDIRPILFPDNQTLQFCNQTPPHLVGPIRVFLDEPDFKTLEKIYPDTHAGGHGMPKDCVARHRVAIIVPYRDREAHLRIMLHNLHSLLAKQQLDYAIFIVEQVANQTFNRGKLMNVGYDVASRLYPWQCFIFHDVDLLPEDDRNLYTCPIQPRHMSVAIDKFNYKLPYSAAFGGISALTKDHLKKINGFSNDFWGWGGEDDDLATRTSMAGLKVSRYPTQIARYKMIKHSTEATNPVNKCRYKIMGQTKRRWTRDGLSNLKYKLVNLELKPLYTRAVVDLLEKDCRRELRRDFPTCF

SEQ ID NO: 13 - protein, 354 aa, synthetic construct
  REGION 1..354: note = CeGalNacT(30-383; M312H)
KIPSLYENLTIGSSTLIADVDAMEAVLGNTASTSDDLLDTWNSTFSPISEVNQTSFMEDIRPILFPDNQTLQFCNQTPPHLVGPIRVFLDEPDFKTLEKIYPDTHAGGHGMPKDCVARHRVAIIVPYRDREAHLRIMLHNLHSLLAKQQLDYAIFIVEQVANQTFNRGKLMNVGYDVASRLYPWQCFIFHDVDLLPEDDRNLYTCPIQPRHMSVAIDKFNYKLPYSAIFGGISALTKDHLKKINGFSNDFWGWGGEDDDLATRTSMAGLKVSRYPTQIARYKHIKHSTEATNPVNKCRYKIMGQTKRRWTRDGLSNLKYKLVNLELKPLYTRAVVDLLEKDCRRELRRDFPTCF

SEQ ID NO: 14 - protein, 360 aa, synthetic construct
  REGION 1..360: note = CeGalNAcT(30-383)-His
KIPSLYENLTIGSSTLIADVDAMEAVLGNTASTSDDLLDTWNSTFSPISEVNQTSFMEDIRPILFPDNQTLQFCNQTPPHLVGPIRVFLDEPDFKTLEKIYPDTHAGGHGMPKDCVARHRVAIIVPYRDREAHLRIMLHNLHSLLAKQQLDYAIFIVEQVANQTFNRGKLMNVGYDVASRLYPWQCFIFHDVDLLPEDDRNLYTCPIQPRHMSVAIDKFNYKLPYSAIFGGISALTKDHLKKINGFSNDFWGWGGEDDDLATRTSMAGLKVSRYPTQIARYKMIKHSTEATNPVNKCRYKIMGQTKRRWTRDGLSNLKYKLVNLELKPLYTRAVVDLLEKDCRRELRRDFPTCFHHHHHH

SEQ ID NO: 15 - protein, 383 aa, Caenorhabditis remanei
MALRHLAVAKLKTFFVLCAALLLVHTMIYKAPSLYENFSIGSSTLIADVDAMEAVLGNTASTSYDLLDTWNSTFSPISEVNQTSFLEDVRPILFTDNQTKPFCNQTPPHLVGPIRVFLDEPDFATLEKIYPDVHTGGHGIPDECIARHRVAVIVPYRDREAHLRIMLHNLHSLLAKQQLDYAIIVVEQIVNQTFNRGKLMNVGYDVASRLYPWQCFIFHDVDLLPEDDRNLYTCPIQPRHMSVAIDKFDYKLPYSTIFGGISALTQEHVKKINGFSNDFWGWGGEDDDLATRTSMAGLKVSRYPAQIARYKMIKHSTEATNPVNKCRYKIMGQTKRRWTRDGLSSLKYKLVKLDLKPLYTRAVVDLLEKDCRRELRKDFPTCF

SEQ ID NO: 16 - protein, 384 aa, Caenorhabditis briggsae
MAFRHLASAKLKTFFVLCAALLLVHAMIYKVPSLYENFSIGSSTLIADVDAMEAVLGNTASTSDDPFDVWNSTFSPISEVNQTAFMEDIRPILFGDANETRPHCNQTPPHLVGPIRVFLDEPDFATLEKIYPETHPGGHGIPTECVARHRVAIIVPYRDREAHLRIMLHNLHSLLAKQQLDYAIFVVEQVANQTFNRGKLMNVGYDVASRLYPWQCFIFHDVDLLPEDDRNLYTCPIQPRHMSVAIDKFHYKLPYSAIFGGISALTQEHVKAINGFSNDFWGWGGEDDDLATRTSQAGLKVSRYPAQIARYKMIKHSTEATNPVNKCRYKIMGQTKRRWKTDGLSSLKYKLVKLELKPLYTRAVVDLLEKECRRELRRDFPTCF

SEQ ID NO: 17 - protein, 464 aa, Wuchereria bancrofti
MPAAGRFVIILLIFGAAAHIFLGGGLSFISDYHIWRPVVESSRQEIVLVHNIDNNSDQNAEKIISNNETKFHLTSATPIDNLVSIHSNFYELFINGLRFGKLTTVYPIINQSINNGSTTDKSTETYAESVYFLKTDGNIHSNTLLSTITDAQSTRQLFGNETLSACNVIPSFQMMHQNLSLVNCPVTPPGLVGPIKVWYDEPTFEEIERLNPNLEAGGHGKPENCLSRHRVAVIVPYRDREAHLRILLHNLHSLLTKQQLDYGIFVIEQHENETFNRAKLMNVGYVEALKLYDWQCFVFHDVDLLAEDDRNIYSCPDQPRHMSVAVNKFKYKLPYGSIFGGVSAIRTEQFATLNGFSNSYWGWGGEDDDLSMRVTSAGYKIMRYPSEIARYQMVQHKSEMKNPINRCRYDLLAKTKVRQQTDGISSLKYECYDLQFFTLFTHIKVKLFEQESKAQLREEGFKRC

SEQ ID NO: 18 - protein, 291 aa, Loa loa
MERQNLSLVDCPIIPPGLVGPIKVWYDEPTFEEIERLNPYLELGGHGKPGSCLSRHRVAIIVPYRDREAHLRILLHNLHSLLTKQQLDYAIFVIEQHENETFNRAKLMNVGYTEAMKLYDWQCFIFHDVDLLAEDDRNIYSCPDQPRHMSVAINKFKYRLPYGSIFGGVSAIRTEQFLKMNGFSNSYWGWGGEDDDLSIRVTSLGYKIMRYPLEIARYQMVKHESETKNPINRCRYDLLAKTKVRQQMDGISSLKYECYDLHFLPLFTHIKVKLFEQESKAQLREEGFKKC

SEQ ID NO: 19 - protein, 296 aa, Cerapachys biroi
MPIRNLAGNGGTARELPVANTTSNATIPRCPLIPPNLVGPVAVSKSPPPLSEMERSFVEVKAGGKGRPADCVARHRVAIIIPFRDRPQHLQTLLYNLHPILLRQQIDYQIFVIEQEGTGTFNRAMLMNVGYVEALKERIFDCFIFHDVDLLPEDDRNLYTCPEQPRHMSVAVDKFKYRLPYADLFGGVSAMSREHFQLVNGFSNVFWGWGGEDDDMANRIKAHGLHISRYPANVARYKMLTHKKEKANPKRYEFLKTGKKRFSTDGLANLQYELCDKRKPKLYTWLLVRLTPPQPS

SEQ ID NO: 20 - protein, 422 aa, Zootermopsis nevadensis
MRCRCLSAWSRITQHVPRQPCLHIHSHLCKVVIVLAVLIALQFLLTTIFEARQIEPLFTVNFTYSGRRSRWGLISHSRGLLSPSHNSSFNGSMRVSVERTLSPVENISGETKNLSFLHTHENAVRNASSLVLNISLPSDLNPTTSPSLTVPFTGKSLCPPIPPNLNGPIKVLKDSPSLEELEKMFPLLEPGGHYHPEECQARDRVAIIVPYRDRAEHLSTFLLNLHPLLQRQQLDYGMFVIEQGGDGPFNRAMLMNVGFVEALKLYSYDCFIFHDVDLLPEDDRNLYTCPEQPRHMSVAVDVLKYKLPYQAIFGGVSAMTKTQFQKVNGFSNLFWGWGGEDDDMSNRVRHHGYHISRYPANIARYKMLAHRKQHANPKRYEFLNTGRKRFKTDGLSNLQYDRKELNLGKLYTRVLVELATPS

SEQ ID NO: 21 - protein, 295 aa, Camponotus floridanus
MPTRNLVGGGTARELPVANATNNTTMPRCPLIPPNLVGPMVVSKSPPPLSEMERSFVEVNAGGRGRPADCVARHRVAIIIPFRDRPQHLQTLLYNLHPILLRQQIEYQIFVIEQEGTGAFNRAMLMNVGYVEALKERTFDCFIFHDVDLLPEDDRNLYTCPEQPRHMSVAVDKFKYRLPYTDLFGGVSAMSREHFQLVNGFSNVFWGWGGEDDDMANRIKAHGLHISRYPANVARYKMLTHKKEKANPKRYEFLKTGKKRFSTDGLANLQYELSDKRKPKLYTWLLVRLTPPQPS

SEQ ID NO: 22 - protein, 310 aa, Crassostrea gigas
MDRGCKPMRVCSSSPSDLVGSLATYKEAPSYKEMIKIYPLVRPGGLYTPPDCIARERVAIIIPFRDREEHLRILLHNLHPMLQRQQLDYGIYVVEQENGTQFNRAMLMNIGYAESIKLYNYTCFIFHDVDLIPENDRIMYDCRDSPRHLSSAVDKFKYKLPYPQLFGGVTAIKRAHFEKVNGHSNKFFGWGGEDDDMFRRLVNNGFKISRYQASLSKYKMIKHLHDAGNKANKRRHHLIKTGKGRYRRDGINNLHYKKLGIEYQYLHTRILVSINETKVMTVSLLYMYSSTTVYIIVNIYTIYCKSRNIR

SEQ ID NO: 23 - protein, 338 aa, Danaus plexippus
MAKKLLTQGTESVTNYTHTTNSSNKNPAKETFNMTKPNLSDDTSTPLLITKIMESIKNLVTTEEDFRDEPSLPLCDEMPPDLGPISVNKTEIELDWVEKRYPEVRSGGIYSSSNCTARHRVAIIVPYRDRQQHLAIFLNHMHPFLMKQQIEYGIYIIEQEGTSEFNRAKLMNVGFVESQRQRSWQCFIFHDIDLLPLDSRNMYSCPKQPRHMSASIDKLNFRLPYEDIFGGVSAMTLEQFTKVNGFSNKYWGWGGEDDDMFYRLKKMNYHIARYKMSIARYAMLDHKKSAPNPKRYQLLSQTSKTFQKDGLSTLEYEVIKVTANHLYTHILVNIDERS

SEQ ID NO: 24 - protein, 941 aa, synthetic construct
  REGION 1..941: note = HuGalNAcT (57-998)
RYGSWRELAKALASRNIPAVDPHLQFYHPQRLSLEDHDIDQGVSSNSSYLKWNKPVPWLSEFRGRANLHVFEDWCGSSIQQLRRNLHFPLYPHIRTTLRKLAVSPKWTNYGLRIFGYLHPFTDGKIQFAIAADDNAEFWLSLDDQVSGLQLLASVGKTGKEWTAPGEFGKFRSQISKPVSLSASHRYYFEVLHKQNEEGTDHVEVAWRRNDPGAKFTIIDSLSLSLFTNETFLQMDEVGHIPQTAASHVDSSNALPRDEQPPADMLRPDPRDTLYRVPLIPKSHLRHVLPDCPYKPSYLVDGLPLQRYQGLRFVHLSFVYPNDYTRLSHMETHNKCFYQENAYYQDRFSFQEYIKIDQPEKQGLEQPGFEENLLEESQYGEVAEETPASNNQNARMLEGRQTPASTLEQDATDYRLRSLRKLLAQPREGLLAPFSKRNSTASFPGRTSHIPVQQPEKRKQKPSPEPSQDSPHSDKWPPGHPVKNLPQMRGPRPRPAGDSPRKTQWLNQVESYIAEQRRGDRMRPQAPGRGWHGEEEVVAAAGQEGQVEGEEEGEEEEEEEDMSEVFEYVPVFDPVVNWDQTFSARNLDFQALRTDWIDLSCNTSGNLLLPEQEALEVTRVFLKKLNQRSRGRYQLQRIVNVEKRQDQLRGGRYLLELELLEQGQRVVRLSEYVSARGWQGIDPAGGEEVEARNLQGLVWDPHNRRRQVLNTRAQEPKLCWPQGFSWSHRAVVHFVVPVKNQARWVQQFIKDMENLFQVTGDPHFNIVITDYSSEDMDVEMALKRSKLRSYQYVKLSGNFERSAGLQAGIDLVKDPHSIIFLCDLHIHFPAGVIDAIRKHCVEGKMAFAPMVMRLHCGATPQWPEGYWEVNGFGLLGIYKSDLDRIGGMNTKEFRDRWGGEDWELLDRILQGLDVERLSLRNFFHHFHSKRGMWSRRQMKTL

SEQ ID NO: 25 - protein, 389 aa, synthetic construct
  REGION 1..389: note = TnGalNAcT(33-421; W336F)
SPLRTYLYTPLYNATQPTLRNVERLAANWPKKIPSNYIEDSEEYSIKNISLSNHTTRASVVHPPSSITETASKLDKNMTIQDGAFAMISPTPLLITKLMDSIKSYVTTEDGVKKAEAVVTLPLCDSMPPDLGPITLNKTELELEWVEKKFPEVEWGGRYSPPNCTARHRVAIIVPYRDRQQHLAIFLNHMHPFLMKQQIEYGIFIVEQEGNKDFNRAKLMNVGFVESQKLVAEGWQCFVFHDIDLLPLDTRNLYSCPRQPRHMSASIDKLHFKLPYEDIFGGVSAMTLEQFTRVNGFSNKYWGFGGEDDDMSYRLKKINYHIARYKMSIARYAMLDHKKSTPNPKRYQLLSQTSKTFQKDGLSTLEYELVQVVQYHLYTHILVNIDERS

SEQ ID NO: 26 - protein, 389 aa, synthetic construct
  REGION 1..389: note = TnGalNAcT(33-421; W336H)
SPLRTYLYTPLYNATQPTLRNVERLAANWPKKIPSNYIEDSEEYSIKNISLSNHTTRASVVHPPSSITETASKLDKNMTIQDGAFAMISPTPLLITKLMDSIKSYVTTEDGVKKAEAVVTLPLCDSMPPDLGPITLNKTELELEWVEKKFPEVEWGGRYSPPNCTARHRVAIIVPYRDRQQHLAIFLNHMHPFLMKQQIEYGIFIVEQEGNKDFNRAKLMNVGFVESQKLVAEGWQCFVFHDIDLLPLDTRNLYSCPRQPRHMSASIDKLHFKLPYEDIFGGVSAMTLEQFTRVNGFSNKYWGHGGEDDDMSYRLKKINYHIARYKMSIARYAMLDHKKSTPNPKRYQLLSQTSKTFQKDGLSTLEYELVQVVQYHLYTHILVNIDERS

SEQ ID NO: 27 - protein, 389 aa, synthetic construct
  REGION 1..389: note = TnGalNAcT(33-421; W336V)
SPLRTYLYTPLYNATQPTLRNVERLAANWPKKIPSNYIEDSEEYSIKNISLSNHTTRASVVHPPSSITETASKLDKNMTIQDGAFAMISPTPLLITKLMDSIKSYVTTEDGVKKAEAVVTLPLCDSMPPDLGPITLNKTELELEWVEKKFPEVEWGGRYSPPNCTARHRVAIIVPYRDRQQHLAIFLNHMHPFLMKQQIEYGIFIVEQEGNKDFNRAKLMNVGFVESQKLVAEGWQCFVFHDIDLLPLDTRNLYSCPRQPRHMSASIDKLHFKLPYEDIFGGVSAMTLEQFTRVNGFSNKYWGVGGEDDDMSYRLKKINYHIARYKMSIARYAMLDHKKSTPNPKRYQLLSQTSKTFQKDGLSTLEYELVQVVQYHLYTHILVNIDERS

SEQ ID NO: 28 - protein, 389 aa, synthetic construct
  REGION 1..389: note = TnGalNAcT(33-421; E339A)
SPLRTYLYTPLYNATQPTLRNVERLAANWPKKIPSNYIEDSEEYSIKNISLSNHTTRASVVHPPSSITETASKLDKNMTIQDGAFAMISPTPLLITKLMDSIKSYVTTEDGVKKAEAVVTLPLCDSMPPDLGPITLNKTELELEWVEKKFPEVEWGGRYSPPNCTARHRVAIIVPYRDRQQHLAIFLNHMHPFLMKQQIEYGIFIVEQEGNKDFNRAKLMNVGFVESQKLVAEGWQCFVFHDIDLLPLDTRNLYSCPRQPRHMSASIDKLHFKLPYEDIFGGVSAMTLEQFTRVNGFSNKYWGWGGADDDMSYRLKKINYHIARYKMSIARYAMLDHKKSTPNPKRYQLLSQTSKTFQKDGLSTLEYELVQVVQYHLYTHILVNIDERS

SEQ ID NO: 29 - protein, 389 aa, synthetic construct
  REGION 1..389: note = TnGalNAcT(33-421; L302A)
SPLRTYLYTPLYNATQPTLRNVERLAANWPKKIPSNYIEDSEEYSIKNISLSNHTTRASVVHPPSSITETASKLDKNMTIQDGAFAMISPTPLLITKLMDSIKSYVTTEDGVKKAEAVVTLPLCDSMPPDLGPITLNKTELELEWVEKKFPEVEWGGRYSPPNCTARHRVAIIVPYRDRQQHLAIFLNHMHPFLMKQQIEYGIFIVEQEGNKDFNRAKLMNVGFVESQKLVAEGWQCFVFHDIDLLPLDTRNLYSCPRQPRHMSASIDKAHFKLPYEDIFGGVSAMTLEQFTRVNGFSNKYWGWGGEDDDMSYRLKKINYHIARYKMSIARYAMLDHKKSTPNPKRYQLLSQTSKTFQKDGLSTLEYELVQVVQYHLYTHILVNIDERS

SEQ ID NO: 30 - protein, 389 aa, synthetic construct
  REGION 1..389: note = TnGalNAcT(33-421; E339D)
SPLRTYLYTPLYNATQPTLRNVERLAANWPKKIPSNYIEDSEEYSIKNISLSNHTTRASVVHPPSSITETASKLDKNMTIQDGAFAMISPTPLLITKLMDSIKSYVTTEDGVKKAEAVVTLPLCDSMPPDLGPITLNKTELELEWVEKKFPEVEWGGRYSPPNCTARHRVAIIVPYRDRQQHLAIFLNHMHPFLMKQQIEYGIFIVEQEGNKDFNRAKLMNVGFVESQKLVAEGWQCFVFHDIDLLPLDTRNLYSCPRQPRHMSASIDKLHFKLPYEDIFGGVSAMTLEQFTRVNGFSNKYWGWGGDDDDMSYRLKKINYHIARYKMSIARYAMLDHKKSTPNPKRYQLLSQTSKTFQKDGLSTLEYELVQVVQYHLYTHILVNIDERS

SEQ ID NO: 31 - protein, 389 aa, synthetic construct
  REGION 1..389: note = TnGalNAcT(33-421; E339S)
SPLRTYLYTPLYNATQPTLRNVERLAANWPKKIPSNYIEDSEEYSIKNISLSNHTTRASVVHPPSSITETASKLDKNMTIQDGAFAMISPTPLLITKLMDSIKSYVTTEDGVKKAEAVVTLPLCDSMPPDLGPITLNKTELELEWVEKKFPEVEWGGRYSPPNCTARHRVAIIVPYRDRQQHLAIFLNHMHPFLMKQQIEYGIFIVEQEGNKDFNRAKLMNVGFVESQKLVAEGWQCFVFHDIDLLPLDTRNLYSCPRQPRHMSASIDKLHFKLPYEDIFGGVSAMTLEQFTRVNGFSNKYWGWGGSDDDMSYRLKKINYHIARYKMSIARYAMLDHKKSTPNPKRYQLLSQTSKTFQKDGLSTLEYELVQVVQYHLYTHILVNIDERS

SEQ ID NO: 32 - protein, 389 aa, synthetic construct
  REGION 1..389: note = TnGalNAcT(33-421; W336H,E339A)
SPLRTYLYTPLYNATQPTLRNVERLAANWPKKIPSNYIEDSEEYSIKNISLSNHTTRASVVHPPSSITETASKLDKNMTIQDGAFAMISPTPLLITKLMDSIKSYVTTEDGVKKAEAVVTLPLCDSMPPDLGPITLNKTELELEWVEKKFPEVEWGGRYSPPNCTARHRVAIIVPYRDRQQHLAIFLNHMHPFLMKQQIEYGIFIVEQEGNKDFNRAKLMNVGFVESQKLVAEGWQCFVFHDIDLLPLDTRNLYSCPRQPRHMSASIDKLHFKLPYEDIFGGVSAMTLEQFTRVNGFSNKYWGHGGADDDMSYRLKKINYHIARYKMSIARYAMLDHKKSTPNPKRYQLLSQTSKTFQKDGLSTLEYELVQVVQYHLYTHILVNIDERS

SEQ ID NO: 33 - protein, 389 aa, synthetic construct
  REGION 1..389: note = TnGalNAcT(33-421; W336H,E339D)
SPLRTYLYTPLYNATQPTLRNVERLAANWPKKIPSNYIEDSEEYSIKNISLSNHTTRASVVHPPSSITETASKLDKNMTIQDGAFAMISPTPLLITKLMDSIKSYVTTEDGVKKAEAVVTLPLCDSMPPDLGPITLNKTELELEWVEKKFPEVEWGGRYSPPNCTARHRVAIIVPYRDRQQHLAIFLNHMHPFLMKQQIEYGIFIVEQEGNKDFNRAKLMNVGFVESQKLVAEGWQCFVFHDIDLLPLDTRNLYSCPRQPRHMSASIDKLHFKLPYEDIFGGVSAMTLEQFTRVNGFSNKYWGHGGDDDDMSYRLKKINYHIARYKMSIARYAMLDHKKSTPNPKRYQLLSQTSKTFQKDGLSTLEYELVQVVQYHLYTHILVNIDERS

SEQ ID NO: 34 - protein, 389 aa, synthetic construct
  REGION 1..389: note = TnGalNAcT(33-421; W336H,E339S)
SPLRTYLYTPLYNATQPTLRNVERLAANWPKKIPSNYIEDSEEYSIKNISLSNHTTRASVVHPPSSITETASKLDKNMTIQDGAFAMISPTPLLITKLMDSIKSYVTTEDGVKKAEAVVTLPLCDSMPPDLGPITLNKTELELEWVEKKFPEVEWGGRYSPPNCTARHRVAIIVPYRDRQQHLAIFLNHMHPFLMKQQIEYGIFIVEQEGNKDFNRAKLMNVGFVESQKLVAEGWQCFVFHDIDLLPLDTRNLYSCPRQPRHMSASIDKLHFKLPYEDIFGGVSAMTLEQFTRVNGFSNKYWGHGGSDDDMSYRLKKINYHIARYKMSIARYAMLDHKKSTPNPKRYQLLSQTSKTFQKDGLSTLEYELVQVVQYHLYTHILVNIDERS

SEQ ID NO: 35 - protein, 389 aa, synthetic construct
  REGION 1..389: note = TnGalNAcT(33-421; L302G)
SPLRTYLYTPLYNATQPTLRNVERLAANWPKKIPSNYIEDSEEYSIKNISLSNHTTRASVVHPPSSITETASKLDKNMTIQDGAFAMISPTPLLITKLMDSIKSYVTTEDGVKKAEAVVTLPLCDSMPPDLGPITLNKTELELEWVEKKFPEVEWGGRYSPPNCTARHRVAIIVPYRDRQQHLAIFLNHMHPFLMKQQIEYGIFIVEQEGNKDFNRAKLMNVGFVESQKLVAEGWQCFVFHDIDLLPLDTRNLYSCPRQPRHMSASIDKGHFKLPYEDIFGGVSAMTLEQFTRVNGFSNKYWGWGGEDDDMSYRLKKINYHIARYKMSIARYAMLDHKKSTPNPKRYQLLSQTSKTFQKDGLSTLEYELVQVVQYHLYTHILVNIDERS

SEQ ID NO: 36 - protein, 389 aa, synthetic construct
  REGION 1..389: note = TnGalNAcT(33-421; I299M)
SPLRTYLYTPLYNATQPTLRNVERLAANWPKKIPSNYIEDSEEYSIKNISLSNHTTRASVVHPPSSITETASKLDKNMTIQDGAFAMISPTPLLITKLMDSIKSYVTTEDGVKKAEAVVTLPLCDSMPPDLGPITLNKTELELEWVEKKFPEVEWGGRYSPPNCTARHRVAIIVPYRDRQQHLAIFLNHMHPFLMKQQIEYGIFIVEQEGNKDFNRAKLMNVGFVESQKLVAEGWQCFVFHDIDLLPLDTRNLYSCPRQPRHMSASMDKLHFKLPYEDIFGGVSAMTLEQFTRVNGFSNKYWGWGGEDDDMSYRLKKINYHIARYKMSIARYAMLDHKKSTPNPKRYQLLSQTSKTFQKDGLSTLEYELVQVVQYHLYTHILVNIDERS

SEQ ID NO: 37 - protein, 389 aa, synthetic construct
  REGION 1..389: note = TnGalNAcT(33-421; I299A)
SPLRTYLYTPLYNATQPTLRNVERLAANWPKKIPSNYIEDSEEYSIKNISLSNHTTRASVVHPPSSITETASKLDKNMTIQDGAFAMISPTPLLITKLMDSIKSYVTTEDGVKKAEAVVTLPLCDSMPPDLGPITLNKTELELEWVEKKFPEVEWGGRYSPPNCTARHRVAIIVPYRDRQQHLAIFLNHMHPFLMKQQIEYGIFIVEQEGNKDFNRAKLMNVGFVESQKLVAEGWQCFVFHDIDLLPLDTRNLYSCPRQPRHMSASADKLHFKLPYEDIFGGVSAMTLEQFTRVNGFSNKYWGWGGEDDDMSYRLKKINYHIARYKMSIARYAMLDHKKSTPNPKRYQLLSQTSKTFQKDGLSTLEYELVQVVQYHLYTHILVNIDERS

SEQ ID NO: 38 - protein, 389 aa, synthetic construct
  REGION 1..389: note = TnGalNAcT(33-421; I299G)
SPLRTYLYTPLYNATQPTLRNVERLAANWPKKIPSNYIEDSEEYSIKNISLSNHTTRASVVHPPSSITETASKLDKNMTIQDGAFAMISPTPLLITKLMDSIKSYVTTEDGVKKAEAVVTLPLCDSMPPDLGPITLNKTELELEWVEKKFPEVEWGGRYSPPNCTARHRVAIIVPYRDRQQHLAIFLNHMHPFLMKQQIEYGIFIVEQEGNKDFNRAKLMNVGFVESQKLVAEGWQCFVFHDIDLLPLDTRNLYSCPRQPRHMSASGDKLHFKLPYEDIFGGVSAMTLEQFTRVNGFSNKYWGWGGEDDDMSYRLKKINYHIARYKMSIARYAMLDHKKSTPNPKRYQLLSQTSKTFQKDGLSTLEYELVQVVQYHLYTHILVNIDERS

SEQ ID NO: 39 - protein, 389 aa, synthetic construct
  REGION 1..389: note = TnGalNAcT(33-421; I311M)
SPLRTYLYTPLYNATQPTLRNVERLAANWPKKIPSNYIEDSEEYSIKNISLSNHTTRASVVHPPSSITETASKLDKNMTIQDGAFAMISPTPLLITKLMDSIKSYVTTEDGVKKAEAVVTLPLCDSMPPDLGPITLNKTELELEWVEKKFPEVEWGGRYSPPNCTARHRVAIIVPYRDRQQHLAIFLNHMHPFLMKQQIEYGIFIVEQEGNKDFNRAKLMNVGFVESQKLVAEGWQCFVFHDIDLLPLDTRNLYSCPRQPRHMSASIDKLHFKLPYEDMFGGVSAMTLEQFTRVNGFSNKYWGWGGEDDDMSYRLKKINYHIARYKMSIARYAMLDHKKSTPNPKRYQLLSQTSKTFQKDGLSTLEYELVQVVQYHLYTHILVNIDERS

SEQ ID NO: 40 - protein, 354 aa, synthetic construct
  REGION 1..354: note = AsGalNAcT(30-383; F248A)
DYSFWSPAFIISAPKTLTTLQPFSQSTSTNDLAVSALESVEFSMLDNSSILHASDNWTNDELVMRAQNENLQLCPMTPPALVGPIKVWMDAPSFAELERLYPFLEPGGHGMPTACRARHRVAIVVPYRDRESHLRTFLHNLHSLLTKQQLDYAIFVVEQTANETFNRAKLMNVGYAEAIRLYDWRCFIFHDVDLLPEDDRNLYSCPDEPRHMSVAVDKANYKLPYGSIFGGISALTREQFEGINGFSNDYWGWGGEDDDLSTRVTLAGYKISRYPAEIARYKMIKHNSEKKNPVNRCRYKLMSATKSRWRNDGLSSLSYDLISLGRLPLYTHIKVDLLEKQSRRYLRTHGFPTC

SEQ ID NO: 41 - protein, 354 aa, synthetic construct
  REGION 1..354: note = AsGalNAcT(30-383; F248G)
DYSFWSPAFIISAPKTLTTLQPFSQSTSTNDLAVSALESVEFSMLDNSSILHASDNWTNDELVMRAQNENLQLCPMTPPALVGPIKVWMDAPSFAELERLYPFLEPGGHGMPTACRARHRVAIVVPYRDRESHLRTFLHNLHSLLTKQQLDYAIFVVEQTANETFNRAKLMNVGYAEAIRLYDWRCFIFHDVDLLPEDDRNLYSCPDEPRHMSVAVDKGNYKLPYGSIFGGISALTREQFEGINGFSNDYWGWGGEDDDLSTRVTLAGYKISRYPAEIARYKMIKHNSEKKNPVNRCRYKLMSATKSRWRNDGLSSLSYDLISLGRLPLYTHIKVDLLEKQSRRYLRTHGFPTC

SEQ ID NO: 42 - protein, 354 aa, synthetic construct
  REGION 1..354: note = AsGalNAcT(30-383; V245M)
DYSFWSPAFIISAPKTLTTLQPFSQSTSTNDLAVSALESVEFSMLDNSSILHASDNWTNDELVMRAQNENLQLCPMTPPALVGPIKVWMDAPSFAELERLYPFLEPGGHGMPTACRARHRVAIVVPYRDRESHLRTFLHNLHSLLTKQQLDYAIFVVEQTANETFNRAKLMNVGYAEAIRLYDWRCFIFHDVDLLPEDDRNLYSCPDEPRHMSVAMDKFNYKLPYGSIFGGISALTREQFEGINGFSNDYWGWGGEDDDLSTRVTLAGYKISRYPAEIARYKMIKHNSEKKNPVNRCRYKLMSATKSRWRNDGLSSLSYDLISLGRLPLYTHIKVDLLEKQSRRYLRTHGFPTC

SEQ ID NO: 43 - protein, 410 aa, synthetic construct
  REGION 1..410: note = His6-TnGalNAcT(33-421; L302A)
MGSSHHHHHHSSGLVPRGSHMSPLRTYLYTPLYNATQPTLRNVERLAANWPKKIPSNYIEDSEEYSIKNISLSNHTTRASVVHPPSSITETASKLDKNMTIQDGAFAMISPTPLLITKLMDSIKSYVTTEDGVKKAEAVVTLPLCDSMPPDLGPITLNKTELELEWVEKKFPEVEWGGRYSPPNCTARHRVAIIVPYRDRQQHLAIFLNHMHPFLMKQQIEYGIFIVEQEGNKDFNRAKLMNVGFVESQKLVAEGWQCFVFHDIDLLPLDTRNLYSCPRQPRHMSASIDKAHFKLPYEDIFGGVSAMTLEQFTRVNGFSNKYWGWGGEDDDMSYRLKKINYHIARYKMSIARYAMLDHKKSTPNPKRYQLLSQTSKTFQKDGLSTLEYELVQVVQYHLYTHILVNIDERS

SEQ ID NO: 44 - protein, 410 aa, synthetic construct
  REGION 1..410: note = His6-TnGalNAcT(33-421; L302G)
MGSSHHHHHHSSGLVPRGSHMSPLRTYLYTPLYNATQPTLRNVERLAANWPKKIPSNYIEDSEEYSIKNISLSNHTTRASVVHPPSSITETASKLDKNMTIQDGAFAMISPTPLLITKLMDSIKSYVTTEDGVKKAEAVVTLPLCDSMPPDLGPITLNKTELELEWVEKKFPEVEWGGRYSPPNCTARHRVAIIVPYRDRQQHLAIFLNHMHPFLMKQQIEYGIFIVEQEGNKDFNRAKLMNVGFVESQKLVAEGWQCFVFHDIDLLPLDTRNLYSCPRQPRHMSASIDKGHFKLPYEDIFGGVSAMTLEQFTRVNGFSNKYWGWGGEDDDMSYRLKKINYHIARYKMSIARYAMLDHKKSTPNPKRYQLLSQTSKTFQKDGLSTLEYELVQVVQYHLYTHILVNIDERS

SEQ ID NO: 45 - protein, 410 aa, synthetic construct
  REGION 1..410: note = His6-TnGalNAcT(33-421; I299M)
MGSSHHHHHHSSGLVPRGSHMSPLRTYLYTPLYNATQPTLRNVERLAANWPKKIPSNYIEDSEEYSIKNISLSNHTTRASVVHPPSSITETASKLDKNMTIQDGAFAMISPTPLLITKLMDSIKSYVTTEDGVKKAEAVVTLPLCDSMPPDLGPITLNKTELELEWVEKKFPEVEWGGRYSPPNCTARHRVAIIVPYRDRQQHLAIFLNHMHPFLMKQQIEYGIFIVEQEGNKDFNRAKLMNVGFVESQKLVAEGWQCFVFHDIDLLPLDTRNLYSCPRQPRHMSASMDKLHFKLPYEDIFGGVSAMTLEQFTRVNGFSNKYWGWGGEDDDMSYRLKKINYHIARYKMSIARYAMLDHKKSTPNPKRYQLLSQTSKTFQKDGLSTLEYELVQVVQYHLYTHILVNIDERS

SEQ ID NO: 46 - protein, 354 aa, synthetic construct
  REGION 1..354: note = AsGalNAcT(30-383; W282H)
DYSFWSPAFIISAPKTLTTLQPFSQSTSTNDLAVSALESVEFSMLDNSSILHASDNWTNDELVMRAQNENLQLCPMTPPALVGPIKVWMDAPSFAELERLYPFLEPGGHGMPTACRARHRVAIVVPYRDRESHLRTFLHNLHSLLTKQQLDYAIFVVEQTANETFNRAKLMNVGYAEAIRLYDWRCFIFHDVDLLPEDDRNLYSCPDEPRHMSVAVDKFNYKLPYGSIFGGISALTREQFEGINGFSNDYWGHGGEDDDLSTRVTLAGYKISRYPAEIARYKMIKHNSEKKNPVNRCRYKLMSATKSRWRNDGLSSLSYDLISLGRLPLYTHIKVDLLEKQSRRYLRTHGFPTC

SEQ ID NO: 47 - protein, 354 aa, synthetic construct
  REGION 1..354: note = AsGalNAcT(30-383; E285D)
DYSFWSPAFIISAPKTLTTLQPFSQSTSTNDLAVSALESVEFSMLDNSSILHASDNWTNDELVMRAQNENLQLCPMTPPALVGPIKVWMDAPSFAELERLYPFLEPGGHGMPTACRARHRVAIVVPYRDRESHLRTFLHNLHSLLTKQQLDYAIFVVEQTANETFNRAKLMNVGYAEAIRLYDWRCFIFHDVDLLPEDDRNLYSCPDEPRHMSVAVDKFNYKLPYGSIFGGISALTREQFEGINGFSNDYWGWGGDDDDLSTRVTLAGYKISRYPAEIARYKMIKHNSEKKNPVNRCRYKLMSATKSRWRNDGLSSLSYDLISLGRLPLYTHIKVDLLEKQSRRYLRTHGFPTC

SEQ ID NO: 48 - protein, 410 aa, synthetic construct
  REGION 1..410: note = His6-TnGalNAcT(33-421; I299A)
MGSSHHHHHHSSGLVPRGSHMSPLRTYLYTPLYNATQPTLRNVERLAANWPKKIPSNYIEDSEEYSIKNISLSNHTTRASVVHPPSSITETASKLDKNMTIQDGAFAMISPTPLLITKLMDSIKSYVTTEDGVKKAEAVVTLPLCDSMPPDLGPITLNKTELELEWVEKKFPEVEWGGRYSPPNCTARHRVAIIVPYRDRQQHLAIFLNHMHPFLMKQQIEYGIFIVEQEGNKDFNRAKLMNVGFVESQKLVAEGWQCFVFHDIDLLPLDTRNLYSCPRQPRHMSASADKLHFKLPYEDIFGGVSAMTLEQFTRVNGFSNKYWGWGGEDDDMSYRLKKINYHIARYKMSIARYAMLDHKKSTPNPKRYQLLSQTSKTFQKDGLSTLEYELVQVVQYHLYTHILVNIDERS

SEQ ID NO: 49 - protein, 410 aa, synthetic construct
  REGION 1..410: note = His6-TnGalNAcT(33-421)
MGSSHHHHHHSSGLVPRGSHMSPLRTYLYTPLYNATQPTLRNVERLAANWPKKIPSNYIEDSEEYSIKNISLSNHTTRASVVHPPSSITETASKLDKNMTIQDGAFAMISPTPLLITKLMDSIKSYVTTEDGVKKAEAVVTLPLCDSMPPDLGPITLNKTELELEWVEKKFPEVEWGGRYSPPNCTARHRVAIIVPYRDRQQHLAIFLNHMHPFLMKQQIEYGIFIVEQEGNKDFNRAKLMNVGFVESQKLVAEGWQCFVFHDIDLLPLDTRNLYSCPRQPRHMSASIDKLHFKLPYEDIFGGVSAMTLEQFTRVNGFSNKYWGWGGEDDDMSYRLKKINYHIARYKMSIARYAMLDHKKSTPNPKRYQLLSQTSKTFQKDGLSTLEYELVQVVQYHLYTHILVNIDERS

SEQ ID NO: 50 - protein, 410 aa, synthetic construct
  REGION 1..410: note = His6-TnGalNAcT(33-421; W336F)
MGSSHHHHHHSSGLVPRGSHMSPLRTYLYTPLYNATQPTLRNVERLAANWPKKIPSNYIEDSEEYSIKNISLSNHTTRASVVHPPSSITETASKLDKNMTIQDGAFAMISPTPLLITKLMDSIKSYVTTEDGVKKAEAVVTLPLCDSMPPDLGPITLNKTELELEWVEKKFPEVEWGGRYSPPNCTARHRVAIIVPYRDRQQHLAIFLNHMHPFLMKQQIEYGIFIVEQEGNKDFNRAKLMNVGFVESQKLVAEGWQCFVFHDIDLLPLDTRNLYSCPRQPRHMSASIDKLHFKLPYEDIFGGVSAMTLEQFTRVNGFSNKYWGFGGEDDDMSYRLKKINYHIARYKMSIARYAMLDHKKSTPNPKRYQLLSQTSKTFQKDGLSTLEYELVQVVQYHLYTHILVNIDERS

SEQ ID NO: 51 - protein, 410 aa, synthetic construct
  REGION 1..410: note = His6-TnGalNAcT(33-421; W336H)
MGSSHHHHHHSSGLVPRGSHMSPLRTYLYTPLYNATQPTLRNVERLAANWPKKIPSNYIEDSEEYSIKNISLSNHTTRASVVHPPSSITETASKLDKNMTIQDGAFAMISPTPLLITKLMDSIKSYVTTEDGVKKAEAVVTLPLCDSMPPDLGPITLNKTELELEWVEKKFPEVEWGGRYSPPNCTARHRVAIIVPYRDRQQHLAIFLNHMHPFLMKQQIEYGIFIVEQEGNKDFNRAKLMNVGFVESQKLVAEGWQCFVFHDIDLLPLDTRNLYSCPRQPRHMSASIDKLHFKLPYEDIFGGVSAMTLEQFTRVNGFSNKYWGHGGEDDDMSYRLKKINYHIARYKMSIARYAMLDHKKSTPNPKRYQLLSQTSKTFQKDGLSTLEYELVQVVQYHLYTHILVNIDERS

SEQ ID NO: 52 - protein, 410 aa, synthetic construct
  REGION 1..410: note = His6-TnGalNAcT(33-421; W336V)
MGSSHHHHHHSSGLVPRGSHMSPLRTYLYTPLYNATQPTLRNVERLAANWPKKIPSNYIEDSEEYSIKNISLSNHTTRASVVHPPSSITETASKLDKNMTIQDGAFAMISPTPLLITKLMDSIKSYVTTEDGVKKAEAVVTLPLCDSMPPDLGPITLNKTELELEWVEKKFPEVEWGGRYSPPNCTARHRVAIIVPYRDRQQHLAIFLNHMHPFLMKQQIEYGIFIVEQEGNKDFNRAKLMNVGFVESQKLVAEGWQCFVFHDIDLLPLDTRNLYSCPRQPRHMSASIDKLHFKLPYEDIFGGVSAMTLEQFTRVNGFSNKYWGVGGEDDDMSYRLKKINYHIARYKMSIARYAMLDHKKSTPNPKRYQLLSQTSKTFQKDGLSTLEYELVQVVQYHLYTHILVNIDERS

SEQ ID NO: 53 - protein, 410 aa, synthetic construct
  REGION 1..410: note = His6-TnGalNAcT(33-421; E339A)
MGSSHHHHHHSSGLVPRGSHMSPLRTYLYTPLYNATQPTLRNVERLAANWPKKIPSNYIEDSEEYSIKNISLSNHTTRASVVHPPSSITETASKLDKNMTIQDGAFAMISPTPLLITKLMDSIKSYVTTEDGVKKAEAVVTLPLCDSMPPDLGPITLNKTELELEWVEKKFPEVEWGGRYSPPNCTARHRVAIIVPYRDRQQHLAIFLNHMHPFLMKQQIEYGIFIVEQEGNKDFNRAKLMNVGFVESQKLVAEGWQCFVFHDIDLLPLDTRNLYSCPRQPRHMSASIDKLHFKLPYEDIFGGVSAMTLEQFTRVNGFSNKYWGWGGADDDMSYRLKKINYHIARYKMSIARYAMLDHKKSTPNPKRYQLLSQTSKTFQKDGLSTLEYELVQVVQYHLYTHILVNIDERS

SEQ ID NO: 54 - protein, 410 aa, synthetic construct
  REGION 1..410: note = His6-TnGalNAcT(33-421; I299G)
MGSSHHHHHHSSGLVPRGSHMSPLRTYLYTPLYNATQPTLRNVERLAANWPKKIPSNYIEDSEEYSIKNISLSNHTTRASVVHPPSSITETASKLDKNMTIQDGAFAMISPTPLLITKLMDSIKSYVTTEDGVKKAEAVVTLPLCDSMPPDLGPITLNKTELELEWVEKKFPEVEWGGRYSPPNCTARHRVAIIVPYRDRQQHLAIFLNHMHPFLMKQQIEYGIFIVEQEGNKDFNRAKLMNVGFVESQKLVAEGWQCFVFHDIDLLPLDTRNLYSCPRQPRHMSASGDKLHFKLPYEDIFGGVSAMTLEQFTRVNGFSNKYWGWGGEDDDMSYRLKKINYHIARYKMSIARYAMLDHKKSTPNPKRYQLLSQTSKTFQKDGLSTLEYELVQVVQYHLYTHILVNIDERS

SEQ ID NO: 55 - protein, 410 aa, synthetic construct
  REGION 1..410: note = His6-TnGalNAcT(33-421; E339D)
MGSSHHHHHHSSGLVPRGSHMSPLRTYLYTPLYNATQPTLRNVERLAANWPKKIPSNYIEDSEEYSIKNISLSNHTTRASVVHPPSSITETASKLDKNMTIQDGAFAMISPTPLLITKLMDSIKSYVTTEDGVKKAEAVVTLPLCDSMPPDLGPITLNKTELELEWVEKKFPEVEWGGRYSPPNCTARHRVAIIVPYRDRQQHLAIFLNHMHPFLMKQQIEYGIFIVEQEGNKDFNRAKLMNVGFVESQKLVAEGWQCFVFHDIDLLPLDTRNLYSCPRQPRHMSASIDKLHFKLPYEDIFGGVSAMTLEQFTRVNGFSNKYWGWGGDDDDMSYRLKKINYHIARYKMSIARYAMLDHKKSTPNPKRYQLLSQTSKTFQKDGLSTLEYELVQVVQYHLYTHILVNIDERS

SEQ ID NO: 56 - protein, 410 aa, synthetic construct
  REGION 1..410: note = His6-TnGalNAcT(33-421; E339S)
MGSSHHHHHHSSGLVPRGSHMSPLRTYLYTPLYNATQPTLRNVERLAANWPKKIPSNYIEDSEEYSIKNISLSNHTTRASVVHPPSSITETASKLDKNMTIQDGAFAMISPTPLLITKLMDSIKSYVTTEDGVKKAEAVVTLPLCDSMPPDLGPITLNKTELELEWVEKKFPEVEWGGRYSPPNCTARHRVAIIVPYRDRQQHLAIFLNHMHPFLMKQQIEYGIFIVEQEGNKDFNRAKLMNVGFVESQKLVAEGWQCFVFHDIDLLPLDTRNLYSCPRQPRHMSASIDKLHFKLPYEDIFGGVSAMTLEQFTRVNGFSNKYWGWGGSDDDMSYRLKKINYHIARYKMSIARYAMLDHKKSTPNPKRYQLLSQTSKTFQKDGLSTLEYELVQVVQYHLYTHILVNIDERS

SEQ ID NO: 57 - protein, 410 aa, synthetic construct
  REGION 1..410: note = His6-TnGalNAcT(33-421; W336H,E339A)
MGSSHHHHHHSSGLVPRGSHMSPLRTYLYTPLYNATQPTLRNVERLAANWPKKIPSNYIEDSEEYSIKNISLSNHTTRASVVHPPSSITETASKLDKNMTIQDGAFAMISPTPLLITKLMDSIKSYVTTEDGVKKAEAVVTLPLCDSMPPDLGPITLNKTELELEWVEKKFPEVEWGGRYSPPNCTARHRVAIIVPYRDRQQHLAIFLNHMHPFLMKQQIEYGIFIVEQEGNKDFNRAKLMNVGFVESQKLVAEGWQCFVFHDIDLLPLDTRNLYSCPRQPRHMSASIDKLHFKLPYEDIFGGVSAMTLEQFTRVNGFSNKYWGHGGADDDMSYRLKKINYHIARYKMSIARYAMLDHKKSTPNPKRYQLLSQTSKTFQKDGLSTLEYELVQVVQYHLYTHILVNIDERS

SEQ ID NO: 58 - protein, 410 aa, synthetic construct
  REGION 1..410: note = His6-TnGalNAcT(33-421; W336H,E339D)
MGSSHHHHHHSSGLVPRGSHMSPLRTYLYTPLYNATQPTLRNVERLAANWPKKIPSNYIEDSEEYSIKNISLSNHTTRASVVHPPSSITETASKLDKNMTIQDGAFAMISPTPLLITKLMDSIKSYVTTEDGVKKAEAVVTLPLCDSMPPDLGPITLNKTELELEWVEKKFPEVEWGGRYSPPNCTARHRVAIIVPYRDRQQHLAIFLNHMHPFLMKQQIEYGIFIVEQEGNKDFNRAKLMNVGFVESQKLVAEGWQCFVFHDIDLLPLDTRNLYSCPRQPRHMSASIDKLHFKLPYEDIFGGVSAMTLEQFTRVNGFSNKYWGHGGDDDDMSYRLKKINYHIARYKMSIARYAMLDHKKSTPNPKRYQLLSQTSKTFQKDGLSTLEYELVQVVQYHLYTHILVNIDERS

SEQ ID NO: 59 - protein, 410 aa, synthetic construct
  REGION 1..410: note = His6-TnGalNAcT(33-421; W336H,E339S)
MGSSHHHHHHSSGLVPRGSHMSPLRTYLYTPLYNATQPTLRNVERLAANWPKKIPSNYIEDSEEYSIKNISLSNHTTRASVVHPPSSITETASKLDKNMTIQDGAFAMISPTPLLITKLMDSIKSYVTTEDGVKKAEAVVTLPLCDSMPPDLGPITLNKTELELEWVEKKFPEVEWGGRYSPPNCTARHRVAIIVPYRDRQQHLAIFLNHMHPFLMKQQIEYGIFIVEQEGNKDFNRAKLMNVGFVESQKLVAEGWQCFVFHDIDLLPLDTRNLYSCPRQPRHMSASIDKLHFKLPYEDIFGGVSAMTLEQFTRVNGFSNKYWGHGGSDDDMSYRLKKINYHIARYKMSIARYAMLDHKKSTPNPKRYQLLSQTSKTFQKDGLSTLEYELVQVVQYHLYTHILVNIDERS

SEQ ID NO: 60 - protein, 410 aa, synthetic construct
  REGION 1..410: note = His6-TnGalNAcT(33-421; I311M)
MGSSHHHHHHSSGLVPRGSHMSPLRTYLYTPLYNATQPTLRNVERLAANWPKKIPSNYIEDSEEYSIKNISLSNHTTRASVVHPPSSITETASKLDKNMTIQDGAFAMISPTPLLITKLMDSIKSYVTTEDGVKKAEAVVTLPLCDSMPPDLGPITLNKTELELEWVEKKFPEVEWGGRYSPPNCTARHRVAIIVPYRDRQQHLAIFLNHMHPFLMKQQIEYGIFIVEQEGNKDFNRAKLMNVGFVESQKLVAEGWQCFVFHDIDLLPLDTRNLYSCPRQPRHMSASIDKLHFKLPYEDMFGGVSAMTLEQFTRVNGFSNKYWGWGGEDDDMSYRLKKINYHIARYKMSIARYAMLDHKKSTPNPKRYQLLSQTSKTFQKDGLSTLEYELVQVVQYHLYTHILVNIDERS

SEQ ID NO: 61 - DNA, 39 bp, synthetic construct
  misc_feature 1..39: note = primer sequence I299M, fwd
  source 1..39: mol_type = other DNA
gtcacatgtcagccagcatggacaaactgcactttaaac

SEQ ID NO: 62 - DNA, 39 bp, synthetic construct
  misc_feature 1..39: note = primer sequence I299M, rev
  source 1..39: mol_type = other DNA
gtttaaagtgcagtttgtccatgctggctgacatgtgac

SEQ ID NO: 63 - DNA, 41 bp, synthetic construct
  misc_feature 1..41: note = primer sequence I299A, fwd
  source 1..41: mol_type = other DNA
gcgtcacatgtcagccagcgccgacaaactgcactttaaac

SEQ ID NO: 64 - DNA, 41 bp, synthetic construct
  misc_feature 1..41: note = primer sequence I299A, rev
  source 1..41: mol_type = other DNA
gtttaaagtgcagtttgtcggcgctggctgacatgtgacgc

SEQ ID NO: 65 - DNA, 41 bp, synthetic construct
  misc_feature 1..41: note = primer sequence I299G, fwd
  source 1..41: mol_type = other DNA
gcgtcacatgtcagccagcggcgacaaactgcactttaaac

SEQ ID NO: 66 - DNA, 41 bp, synthetic construct
  misc_feature 1..41: note = primer sequence I299G, rev
  source 1..41: mol_type = other DNA
gtttaaagtgcagtttgtcgccgctggctgacatgtgacgc

SEQ ID NO: 67 - DNA, 35 bp, synthetic construct
  misc_feature 1..35: note = primer sequence L302A, fwd
  source 1..35: mol_type = other DNA
cagccagcatcgacaaagcgcactttaaactgccg

SEQ ID NO: 68 - DNA, 35 bp, synthetic construct
  misc_feature 1..35: note = primer sequence L302A, rev
  source 1..35: mol_type = other DNA
cggcagtttaaagtgcgctttgtcgatgctggctg

SEQ ID NO: 69 - DNA, 35 bp, synthetic construct
  misc_feature 1..35: note = primer sequence L302G, fwd
  source 1..35: mol_type = other DNA
cagccagcatcgacaaagggcactttaaactgccg

SEQ ID NO: 70 - DNA, 35 bp, synthetic construct
  misc_feature 1..35: note = primer sequence L302G, rev
  source 1..35: mol_type = other DNA
cggcagtttaaagtgccctttgtcgatgctggctg

SEQ ID NO: 71 - protein, 375 aa, synthetic construct
  REGION 1..375: note = His6-AsGalNAcT(30-383)
MGSSHHHHHHSSGLVPRGSHMDYSFWSPAFIISAPKTLTTLQPFSQSTSTNDLAVSALESVEFSMLDNSSILHASDNWTNDELVMRAQNENLQLCPMTPPALVGPIKVWMDAPSFAELERLYPFLEPGGHGMPTACRARHRVAIVVPYRDRESHLRTFLHNLHSLLTKQQLDYAIFVVEQTANETFNRAKLMNVGYAEAIRLYDWRCFIFHDVDLLPEDDRNLYSCPDEPRHMSVAVDKFNYKLPYGSIFGGISALTREQFEGINGFSNDYWGWGGEDDDLSTRVTLAGYKISRYPAEIARYKMIKHNSEKKNPVNRCRYKLMSATKSRWRNDGLSSLSYDLISLGRLPLYTHIKVDLLEKQSRRYLRTHGFPTC

SEQ ID NO: 72 - protein, 375 aa, synthetic construct
  REGION 1..375: note = His6-AsGalNAcT(30-383; W282H)
MGSSHHHHHHSSGLVPRGSHMDYSFWSPAFIISAPKTLTTLQPFSQSTSTNDLAVSALESVEFSMLDNSSILHASDNWTNDELVMRAQNENLQLCPMTPPALVGPIKVWMDAPSFAELERLYPFLEPGGHGMPTACRARHRVAIVVPYRDRESHLRTFLHNLHSLLTKQQLDYAIFVVEQTANETFNRAKLMNVGYAEAIRLYDWRCFIFHDVDLLPEDDRNLYSCPDEPRHMSVAVDKFNYKLPYGSIFGGISALTREQFEGINGFSNDYWGHGGEDDDLSTRVTLAGYKISRYPAEIARYKMIKHNSEKKNPVNRCRYKLMSATKSRWRNDGLSSLSYDLISLGRLPLYTHIKVDLLEKQSRRYLRTHGFPTC

SEQ ID NO: 73 - protein, 375 aa, synthetic construct
  REGION 1..375: note = His6-AsGalNAcT(30-383; E285D)
MGSSHHHHHHSSGLVPRGSHMDYSFWSPAFIISAPKTLTTLQPFSQSTSTNDLAVSALESVEFSMLDNSSILHASDNWTNDELVMRAQNENLQLCPMTPPALVGPIKVWMDAPSFAELERLYPFLEPGGHGMPTACRARHRVAIVVPYRDRESHLRTFLHNLHSLLTKQQLDYAIFVVEQTANETFNRAKLMNVGYAEAIRLYDWRCFIFHDVDLLPEDDRNLYSCPDEPRHMSVAVDKFNYKLPYGSIFGGISALTREQFEGINGFSNDYWGWGGDDDDLSTRVTLAGYKISRYPAEIARYKMIKHNSEKKNPVNRCRYKLMSATKSRWRNDGLSSLSYDLISLGRLPLYTHIKVDLLEKQSRRYLRTHGFPTC

SEQ ID NO: 74 - DNA, 31 bp, synthetic construct
  misc_feature 1..31: note = primer sequence I311M, fwd
  source 1..31: mol_type = other DNA
cgaagatatgttcggcggtgtctcagccatg

SEQ ID NO: 75 - DNA, 1173 bp, synthetic construct
  misc_feature 1..1173: note = TnGalNAcT(33-421)
  source 1..1173: mol_type = other DNA
atgtcaccgctgcgtacctacctgtataccccgctgtataatgccacccaaccgaccctgcgtaatgtggaacgtctggctgcgaactggccgaagaaaattccgagcaactatatcgaagattcagaagaatactcgatcaaaaacatcagtctgtccaatcataccacgcgtgcgagtgtggttcacccgccgagctctatcaccgaaacggcctccaaactggacaaaaatatgaccattcaggatggcgcgttcgccatgattagcccgaccccgctgctgatcacgaaactgatggacagcattaaatcttatgtcaccacggaagatggcgtgaagaaagcggaagctgtcgttaccctgccgctgtgtgactccatgccgccagatctgggtccgattaccctgaacaaaacggaactggaactggaatgggttgagaaaaaatttccggaagtcgaatggggcggtcgctatagtccgccgaactgtaccgcacgtcatcgcgtggctattatcgttccgtaccgtgaccgccagcaacacctggcaatctttctgaatcacatgcacccgttcctgatgaaacagcaaattgaatacggcatttttatcgtggaacaggaaggtaataaagatttcaatcgtgcaaaactgatgaacgttggctttgtcgaatctcagaaactggtggctgaaggttggcaatgctttgttttccatgacatcgatctgctgccgctggatacccgcaatctgtatagttgtccgcgccagccgcgtcacatgtcagccagcatcgacaaactgcactttaaactgccgtacgaagatattttcggcggtgtctcagccatgaccctggaacaatttacgcgtgttaacggcttctcgaataaatattggggttggggcggtgaagatgacgatatgagctaccgcctgaagaaaattaactatcatatcgcccgttacaaaatgagcattgcgcgctatgccatgctggaccacaaaaaatctaccccgaatccgaaacgttaccagctgctgagtcaaaccagcaaaacgtttcagaaagatggtctgtctacgctggaatatgaactggtccaagttgtgcagtatcatctgtacacgcatattctggtgaacattgacgaacgctcttga

SEQ ID NO: 76 - DNA, 1233 bp, synthetic construct
  misc_feature 1..1233: note = His6-TnGalNAcT(33-421)
  source 1..1233: mol_type = other DNA
atgggcagcagccatcatcatcatcatcacagcagcggcctggtgccgcgcggcagccatatgtcaccgctgcgtacctacctgtataccccgctgtataatgccacccaaccgaccctgcgtaatgtggaacgtctggctgcgaactggccgaagaaaattccgagcaactatatcgaagattcagaagaatactcgatcaaaaacatcagtctgtccaatcataccacgcgtgcgagtgtggttcacccgccgagctctatcaccgaaacggcctccaaactggacaaaaatatgaccattcaggatggcgcgttcgccatgattagcccgaccccgctgctgatcacgaaactgatggacagcattaaatcttatgtcaccacggaagatggcgtgaagaaagcggaagctgtcgttaccctgccgctgtgtgactccatgccgccagatctgggtccgattaccctgaacaaaacggaactggaactggaatgggttgagaaaaaatttccggaagtcgaatggggcggtcgctatagtccgccgaactgtaccgcacgtcatcgcgtggctattatcgttccgtaccgtgaccgccagcaacacctggcaatctttctgaatcacatgcacccgttcctgatgaaacagcaaattgaatacggcatttttatcgtggaacaggaaggtaataaagatttcaatcgtgcaaaactgatgaacgttggctttgtcgaatctcagaaactggtggctgaaggttggcaatgctttgttttccatgacatcgatctgctgccgctggatacccgcaatctgtatagttgtccgcgccagccgcgtcacatgtcagccagcatcgacaaactgcactttaaactgccgtacgaagatattttcggcggtgtctcagccatgaccctggaacaatttacgcgtgttaacggcttctcgaataaatattggggttggggcggtgaagatgacgatatgagctaccgcctgaagaaaattaactatcatatcgcccgttacaaaatgagcattgcgcgctatgccatgctggaccacaaaaaatctaccccgaatccgaaacgttaccagctgctgagtcaaaccagcaaaacgtttcagaaagatggtctgtctacgctggaatatgaactggtccaagttgtgcagtatcatctgtacacgcatattctggtgaacattgacgaacgctcttga

SEQ ID NO: 77 - DNA, 1068 bp, synthetic construct
  misc_feature 1..1068: note = AsGalNAcT(30-383)
  source 1..1068: mol_type = other DNA
atggattactcattctggagcccggcgttcatcatctctgccccgaaaaccctgaccaccctgcaaccgttctctcagtctacctctaccaacgacctggcagtctcagctctggaatcggtggaatttagcatgctggataatagctctattctgcatgcgtctgacaactggaccaatgatgaactggtgatgcgcgcccagaacgaaaatctgcaactgtgtccgatgacgccgccggcgctggttggcccgatcaaagtttggatggatgcgccgagctttgccgaactggaacgtctgtatccgttcctggaaccgggcggtcatggtatgccgaccgcctgtcgtgcacgtcaccgtgttgccattgtggttccgtatcgcgaccgtgaatcccacctgcgcaccttcctgcataacctgcactcactgctgacgaaacagcaactggattacgcaatctttgtcgtggaacagaccgcaaacgaaacgttcaatcgtgctaaactgatgaatgttggctatgcggaagccattcgcctgtacgattggcgttgctttatcttccatgacgtcgatctgctgccggaagatgaccgcaacctgtattcttgtccggacgaaccgcgtcacatgagtgttgcagtcgataaattcaactacaaactgccgtacggttcgattttcggcggtatcagcgctctgacccgcgaacaatttgaaggcattaacggtttcagcaatgattactggggctggggcggtgaagatgacgatctgtcgacccgtgtgacgctggcgggttataaaatcagccgctacccggcagaaatcgctcgttacaaaatgatcaaacataacagtgaaaagaaaaacccggttaatcgctgccgttacaaactgatgtctgccaccaaaagtcgctggcgtaatgacggcctgagttccctgtcctatgatctgatttcactgggtcgcctgccgctgtacacgcacatcaaagttgacctgctggaaaaacaatctcgccgctatctgcgtacccacggcttcccgacctgctga

SEQ ID NO: 78 - DNA, 1128 bp, synthetic construct
  misc_feature 1..1128: note = His6-AsGalNAcT(30-383)
  source 1..1128: mol_type = other DNA
atgggcagcagccatcatcatcatcatcacagcagcggcctggtgccgcgcggcagccatatggattactcattctggagcccggcgttcatcatctctgccccgaaaaccctgaccaccctgcaaccgttctctcagtctacctctaccaacgacctggcagtctcagctctggaatcggtggaatttagcatgctggataatagctctattctgcatgcgtctgacaactggaccaatgatgaactggtgatgcgcgcccagaacgaaaatctgcaactgtgtccgatgacgccgccggcgctggttggcccgatcaaagtttggatggatgcgccgagctttgccgaactggaacgtctgtatccgttcctggaaccgggcggtcatggtatgccgaccgcctgtcgtgcacgtcaccgtgttgccattgtggttccgtatcgcgaccgtgaatcccacctgcgcaccttcctgcataacctgcactcactgctgacgaaacagcaactggattacgcaatctttgtcgtggaacagaccgcaaacgaaacgttcaatcgtgctaaactgatgaatgttggctatgcggaagccattcgcctgtacgattggcgttgctttatcttccatgacgtcgatctgctgccggaagatgaccgcaacctgtattcttgtccggacgaaccgcgtcacatgagtgttgcagtcgataaattcaactacaaactgccgtacggttcgattttcggcggtatcagcgctctgacccgcgaacaatttgaaggcattaacggtttcagcaatgattactggggctggggcggtgaagatgacgatctgtcgacccgtgtgacgctggcgggttataaaatcagccgctacccggcagaaatcgctcgttacaaaatgatcaaacataacagtgaaaagaaaaacccggttaatcgctgccgttacaaactgatgtctgccaccaaaagtcgctggcgtaatgacggcctgagttccctgtcctatgatctgatttcactgggtcgcctgccgctgtacacgcacatcaaagttgacctgctggaaaaacaatctcgccgctatctgcgtacccacggcttcccgacctgctga

SEQ ID NO: 79 - DNA, 43 bp, synthetic construct
  misc_feature 1..43: note = primer sequence W336F, fwd
  source 1..43: mol_type = other DNA
ctcgaataaatattggggttttggcggtgaagatgacgatatg

SEQ ID NO: 80 - DNA, 43 bp, synthetic construct
  misc_feature 1..43: note = primer sequence W336F,rev
  source 1..43: mol_type = other DNA
catatcgtcatcttcaccgccaaaaccccaatatttattcgag

SEQ ID NO: 81 - DNA, 36 bp, synthetic construct
  misc_feature 1..36: note = primer sequence W336H,fwd
  source 1..36: mol_type = other DNA
cgaataaatattggggtcacggcggtgaagatgacg

SEQ ID NO: 82 - DNA, 36 bp, synthetic construct
  misc_feature 1..36: note = primer sequence W336H,rev
  source 1..36: mol_type = other DNA
cgtcatcttcaccgccgtgaccccaatatttattcg

SEQ ID NO: 83 - DNA, 36 bp, synthetic construct
  misc_feature 1..36: note = primer sequence W336V,fwd
  source 1..36: mol_type = other DNA
cgaataaatattggggtgtgggcggtgaagatgacg

SEQ ID NO: 84 - DNA, 36 bp, synthetic construct
  misc_feature 1..36: note = primer sequence W336V, rev
  source 1..36: mol_type = other DNA
cgtcatcttcaccgcccacaccccaatatttattcg

SEQ ID NO: 85 - DNA, 31 bp, synthetic construct
  misc_feature 1..31: note = primer sequence E339A,fwd
  source 1..31: mol_type = other DNA
gggttggggcggtgcggatgacgatatgagc

SEQ ID NO: 86 - DNA, 31 bp, synthetic construct
  misc_feature 1..31: note = primer sequence E339A,rev
  source 1..31: mol_type = other DNA
gctcatatcgtcatccgcaccgccccaaccc

SEQ ID NO: 87 - DNA, 31 bp, synthetic construct
  misc_feature 1..31: note = primer sequence I311M, rev
  source 1..31: mol_type = other DNA
catggctgagacaccgccgaacatatcttcg

SEQ ID NO: 88 - DNA, 31 bp, synthetic construct
  misc_feature 1..31: note = primer sequence E339D,fwd
  source 1..31: mol_type = other DNA
gggttggggcggtgatgatgacgatatgagc

SEQ ID NO: 89 - DNA, 31 bp, synthetic construct
  misc_feature 1..31: note = primer sequence E339D,rev
  source 1..31: mol_type = other DNA
gctcatatcgtcatcatcaccgccccaaccc